European Patent Specification EP 4 032 409 B1, published September 9, 2026. Title: METHODS OF IMPROVING ANIMAL PERFORMANCE. Applicant: DSM IP ASSETS B.V. NOVOZYMES A/S. The sequence listing filed with the application follows.

SEQUENCE LISTING (15 sequences)

SEQ ID NO: 1 - protein, 213 aa, Artificial Sequence
  Wild type sequence with N-terminal SPIRR
SPIRRRIPGFDISGWQPTTDFARAYANGDRFVYIKATEGTTFKSSAFSRQYTGATQNGFIRGAYHFAQPAASSGAAQARYFASNGGGWSKDGITLPGALDIEYNPNGATCYGLSQSAMVNWIEDFVTTYHGITSRWPVIYTTTDWWTQCTGNSNRFANRCPLWIARYASSVGTLPNGWGFYTFWQYNDKYPQGGDSNWFNGDASRLRALANGD

SEQ ID NO: 2 - DNA, 946 bp, Trichophaea saccata
  CDS (1)..(347)
  sig_peptide (1)..(51)
  mat_peptide (52)..(943)
  CDS (401)..(615)
  CDS (668)..(772)
  CDS (825)..(943)
atgcacgctctcacccttctcaccgcaaccctcttcggtctcgcagcggcctacccagtgaagaccgaccttcactgccgctcctctcccagcacttccgccagcatcgtccgcacctactccagtggaacggaagtccagatccagtgccagaccacgggcacttcggtccaaggatccaatgtctgggacaagacccagcacggttgctacgtcgcagactactacgtcaagaccgggcattctgggattttcaccaccaagtgcggtagcagctcgggtggaggttcctgcaagcctcccccgatcaatgctgctactgtcgcattgatcaaggagtttgaggggtaagtgacagctctgagtgaggtggtatgaggattaagactgacgaggatagattcgttcctaagcccgccccggatcctattggattgccgaccgtgggatacgggcatctttgcaagactaagggctgcaaagaagtgccttacagcttccctctcacccaggagactgccaccaagttgcttcagagcgatatcaagactttcacctcttgcgttagcaactacgtcaaggactctgttaagctcaacgataaccagtacggaggtgagttccagtgtaacagtgaatttattgatgatattctaagtaattttagctctggcgtcttgggctttcaacgtcggctgcggaaacgtccagacttcttcgctgatcaagagattgaacgctggggagaaccctaacactgtcgctgctcagggtaagatatttatcccggatttgctcttgacacatggctgaaaaagttgcagaactccccaagtggaagtacgctggtggaaaggttatgcctggcttggtccgccgccgcaatgctgaggtcgcgctcttcaagaagcccagcagcgttcaggcccaccctcccaagtgctaa

SEQ ID NO: 3 - protein, 262 aa, Trichophaea saccata
MHALTLLTATLFGLAAAYPVKTDLHCRSSPSTSASIVRTYSSGTEVQIQCQTTGTSVQGSNVWDKTQHGCYVADYYVKTGHSGIFTTKCGSSSGGGSCKPPPINAATVALIKEFEGFVPKPAPDPIGLPTVGYGHLCKTKGCKEVPYSFPLTQETATKLLQSDIKTFTSCVSNYVKDSVKLNDNQYGALASWAFNVGCGNVQTSSLIKRLNAGENPNTVAAQELPKWKYAGGKVMPGLVRRRNAEVALFKKPSSVQAHPPKC

SEQ ID NO: 4 - protein, 245 aa, Trichophaea saccata
  mat_peptide (1)..(245)
YPVKTDLHCRSSPSTSASIVRTYSSGTEVQIQCQTTGTSVQGSNVWDKTQHGCYVADYYVKTGHSGIFTTKCGSSSGGGSCKPPPINAATVALIKEFEGFVPKPAPDPIGLPTVGYGHLCKTKGCKEVPYSFPLTQETATKLLQSDIKTFTSCVSNYVKDSVKLNDNQYGALASWAFNVGCGNVQTSSLIKRLNAGENPNTVAAQELPKWKYAGGKVMPGLVRRRNAEVALFKKPSSVQAHPPKC

SEQ ID NO: 5 - protein, 129 aa, Gallus gallus [sequence omitted]

SEQ ID NO: 6 - DNA, 39 bp, Artificial Sequence
  Primer F-80470
acacaactggggatccaccatgcacgctctcacccttct

SEQ ID NO: 7 - DNA, 38 bp, Artificial Sequence
  Primer R-80470.
ctagatctcgagaagcttttagcacttgggagggtggg

SEQ ID NO: 8 - DNA, 20 bp, Artificial Sequence
  Primer 8643.
gcaagggatgccatgcttgg

SEQ ID NO: 9 - DNA, 19 bp, Artificial Sequence
  Primer 8654.
catataaccaattgccctc

SEQ ID NO: 10 - DNA, 20 bp, Artificial Sequence
  Forward primer 27F.
agagtttgatcctggctcag

SEQ ID NO: 11 - DNA, 17 bp, Artificial Sequence
  Reverse primer 534R.
attaccgcggctgctgg

SEQ ID NO: 12 - protein, 213 aa, Acremonium alcalophilum; identical to SEQ ID NO: 1

SEQ ID NO: 13 - DNA, 470 bp, Faecalibacterium sp.
gacgaacgctggcggcgcgcctaacacatgcaagtcgaacggaatgcggagaggatttatcttttctgtgtttagtggcgaacgggtgagtaacgcgtgaggaacctgcctcaaagagggggacaacagttggaaacgactgctaataccgcataagcccacggggccgcatggctctgagggaaaaggagcaatccgctttgagatggcctcgcgtccgattagctggttggtgaggtaacggcccaccaaggcgacgatcggtagccggactgagaggttgaacggccacattgggactgagacacggcccagactcctacgggaggcagcagtggggaatattgcacaatgggggaaaccctgatgcagcgacgccgcgtggaggaagaaggtcttcggattgtaaactcctgttgttggggaaaagaaggatggtacccaacaaggaagtgacggctaactacgtg

SEQ ID NO: 14 - DNA, 468 bp, Faecalibacterium sp.
gacgaacgctggcggcgcgcctaacacatgcaagtcgaacggagttgagaggagcttgcttttcttgacttagtggcgaacgggtgagtaacgcgtgaggaacctgcctcaaagagggggacaacagttggaaacgactgctaataccgcataagcccacggtcccgcatgggagagagggaaaaggagcaatccgctttgagatggcctcgcgtccgattagctagttggtgaggtaacggcccaccaaggcgacgatcggtagccggactgagaggttgaacggccacattgggactgagacacggcccagactcctacgggaggcagcagtggggaatattgcacaatgggggaaaccctgatgcagcgacgccgcgtggaggaagaaggtcttcggattgtaaactcctgttgttggggaaaaagaggatggtacccaacaaggaagtgacggctaactacgtg

SEQ ID NO: 15 - DNA, 468 bp, Faecalibacterium sp.
gacgaacgctggcggcgcgcctaacacatgcaagtcgaacggagcttgagggagcttgcttctttaagcttagtggcgaacgggtgagtaacgcgtgaggaacctgcctcagagtgggggacaacagttggaaacgactgctaataccgcataagcccacggatccgcatggatctgagggaaaaggagcaatccgctttgagatggcctcgcgtccgattagctggttggtgaggtaacggcccaccaaggcgacgatcggtagccggactgagaggttgaacggccacattgggactgagacacggcccagactcctacgggaggcagcagtggggaatattgcacaatgggggaaaccctgatgcagcgacgccgcgtggaggaagaaggtcttcggattgtaaactcctgttgttagggaaaatcgagatggtacctaacaaggaagtgacggctaactacgtg